European Patent Specification EP 3 394 282 B1, published June 7, 2023. Title: Production of sterols in modified yeast. Applicant: DSM IP Assets B.V. The sequence listing filed with the application follows.

SEQUENCE LISTING (37 sequences)

SEQ ID NO: 1 - DNA, 40 bp, Artificial Sequence
  primer
ctatatggatccaaaatgacggagactaaggatttgttgc

SEQ ID NO: 2 - DNA, 40 bp, Artificial Sequence
  primer
gactgcgaattctcataaggtcaggtacaacgtcataatg

SEQ ID NO: 3 - DNA, 24 bp, Artificial Sequence
  primer
gtggcgggtatccagccgccgaag

SEQ ID NO: 4 - DNA, 24 bp, Artificial Sequence
  primer
cttcggcggctggatacccgccac

SEQ ID NO: 5 - DNA, 40 bp, Artificial Sequence
  primer
ctatatggatccaaaatggacaagaagaaggatctactgg

SEQ ID NO: 6 - DNA, 40 bp, Artificial Sequence
  primer
gactgcgaattcttagaatgtcaagtacaacgtacacatg

SEQ ID NO: 7 - DNA, 73 bp, Artificial Sequence
  primer
cataatttaaaaaaacaagaataaaataataatatagtaggcagcataagatgtctgttattaatttcacagg

SEQ ID NO: 8 - DNA, 72 bp, Artificial Sequence
  primer
ataggtatatatcgtgcgctttatttgaatcttattgatctagtgaatttctatttcttagcatttttgacg

SEQ ID NO: 9 - DNA, 71 bp, Artificial Sequence
  primer
aaaacatcacattttgctattccaatagacaataaataccttttaacaaaatgtctgcccctaagaagatc

SEQ ID NO: 10 - DNA, 74 bp, Artificial Sequence
  primer
taatgaagtaaatatgatttattgtctggacaaagttctgtttttccccattaagcaaggattttcttaacttc

SEQ ID NO: 11 - DNA, 64 bp, Artificial Sequence
  primer
ctataaagatttaatagctccacagaacagttgcaggatgccgcataggccactagtggatctg

SEQ ID NO: 12 - DNA, 64 bp, Artificial Sequence; identical to SEQ ID NO: 11
  primer

SEQ ID NO: 13 - DNA, 63 bp, Artificial Sequence
  primer
atgacggagactaaggatttgttgcaagacgaagagtttcttaaagcttgcctcgtccccgcc

SEQ ID NO: 14 - DNA, 65 bp, Artificial Sequence
  primer
tcataaggtcaggtacaacgtcataatgatactgggccctgaactggatggcggcgttagtatcg

SEQ ID NO: 15 - DNA, 47 bp, Artificial Sequence
  primer
gttgttggatccaaaaatgatggcttcagatagagttagaaaaagac

SEQ ID NO: 16 - DNA, 44 bp, Artificial Sequence
  primer
caacaagaattctcatcagaaaatatttggcaataatctataag

SEQ ID NO: 17 - DNA, 89 bp, Artificial Sequence
  primer
aaaacatcacattttgctattccaatagacaataaataccttttaacaaaagtttatcattatcaatactcgccatttcaaagaatacg

SEQ ID NO: 18 - DNA, 73 bp, Artificial Sequence
  primer
taatgaagtaaatatgatttattgtctggacaaagttctgtttttccccaggccgcaaattaaagccttcgag

SEQ ID NO: 19 - DNA, 62 bp, Artificial Sequence
  primer
gcgggatccatggactacaaagacgatgacgataaagtcggagaggaaaagatgtccctgac

SEQ ID NO: 20 - DNA, 62 bp, Artificial Sequence
  primer
gcggaattctcagaaaacgtaacgacaagtccatgatctaggcctaacgtaatccagaaagg

SEQ ID NO: 21 - DNA, 62 bp, Artificial Sequence
  primer
gcgggatccatggactacaaagacgatgacgataaagaaccaaaagctccacaattacgtcg

SEQ ID NO: 22 - DNA, 71 bp, Artificial Sequence
  primer
gcggaattctcaaggatgacaactccaggatctaggtgttacaagttcccaaaatgttggttgtggtaatg

SEQ ID NO: 23 - DNA, 63 bp, Artificial Sequence
  primer
gcgggatccatggactacaaagacgatgacgataaaggatccaaaatggtaggcgaggaaatg

SEQ ID NO: 24 - DNA, 78 bp, Artificial Sequence
  primer
gcggaattctcaaaacacatatctacaagtccatgtacgtggtctgacgtaatcaaggaaagtagggtttttcaatgg

SEQ ID NO: 25 - DNA, 61 bp, Artificial Sequence
  primer
gcgggatccatggactacaaagacgatgacgataaaggcagaactaacacttctgatcagc

SEQ ID NO: 26 - DNA, 81 bp, Artificial Sequence
  primer$
gcggaattctcaaaagaccaggtacagagtacagataatggaagggccagagatgaaaccgaaccaacaaatgatgttacc

SEQ ID NO: 27 - DNA, 62 bp, Artificial Sequence
  primer
gcgggatccatggactacaaagacgatgacgataaattagatgatcctttgtctaaaactag

SEQ ID NO: 28 - DNA, 70 bp, Artificial Sequence
  primer
gcggaattctctcaaaacaatcttaaaggttgatgatcggcatgagcattgtaaaagtgtatttgtgccc

SEQ ID NO: 29 - DNA, 60 bp, Artificial Sequence
  primer
gcgggatccaaaatggactacaaagacgatgacgataaaacggagactaaggatttgttg

SEQ ID NO: 30 - DNA, 59 bp, Artificial Sequence
  primer
gctgaattctcataaggtcaggtacaacgtcataatgatactgggccctgaacagacac

SEQ ID NO: 31 - DNA, 60 bp, Artificial Sequence
  primer
gcgggatccatggactacaaagacgatgacgataaagacaagaagaaggatctactggag

SEQ ID NO: 32 - DNA, 60 bp, Artificial Sequence
  primer
gcggaattcttagaatgtcaagtacaacgtacacatgacacttggtcccatgcagatacc

SEQ ID NO: 33 - DNA, 33 bp, Artificial Sequence
  primer
aacactacatatgcgtatatataccaatctaag

SEQ ID NO: 34 - DNA, 39 bp, Artificial Sequence
  primer
ggtggtgcggccgccacagatgcgtaaggagaaaatacc

SEQ ID NO: 35 - DNA, 29 bp, Artificial Sequence
  primer
ggtggtcatatgagcttgcctcgtccccg

SEQ ID NO: 36 - DNA, 34 bp, Artificial Sequence
  primer
ggtggtgcggccgcggatggcggcgttagtatcg

SEQ ID NO: 37 - DNA, 40 bp, Artificial Sequence
  primer
cgcggatccgcgaaaatggactacaaagacgatgacgata